European Patent Specification EP 3 663 313 B1, published April 3, 2024. Title: N-terminal recombinant protein of CCR4 and usage thereof. Applicant: Institute of Biophysics, Chinese Academy of Sciences. Application EP18907350.5. The sequence listing filed with the application follows.

SEQUENCE LISTING (7 sequences)

SEQ ID NO: 1 - protein, 47 aa, Artificial
  N-CCR4 protein
MNPTDIADTTLDESIYSNYYLYESIPKPCTKEGIKAFGELFLPPLYS

SEQ ID NO: 2 - protein, 183 aa, Artificial
  (N-CCR4)3 protein
MNPTDIADTTLDESIYSNYYLYESIPKPCTKEGIKAFGELFLPPLYSGGGGSGGGGSMNPTDIADTTLDESIYSNYYLYESIPKPCTKEGIKAFGELFLPPLYSGGGGSGGGGSMNPTDIADTTLDESIYSNYYLYESIPKPCTKEGIKAFGELFLPPLYSLDPNSSSVDKLAAALEHHHHHH

SEQ ID NO: 3 - protein, 390 aa, Artificial
  (N-CCR4)3-Fc protein
MNPTDIADTTLDESIYSNYYLYESIPKPCTKEGIKAFGELFLPPLYSGGGGSGGGGSMNPTDIADTTLDESIYSNYYLYESIPKPCTKEGIKAFGELFLPPLYSGGGGSGGGGSMNPTDIADTTLDESIYSNYYLYESIPKPCTKEGIKAFGELFLPPLYSKLDKTHTCPPCPAPELLGGPSVFLFPPKPKDTLMISRTPEVTCVVVDVSHEDPEVKFNWYVDGVEVHNAKTKPREEQYNSTYRVVSVLTVLHQDWLNGKEYKCKVSNKALPAPIEKTISKAKGQPREPQVYTLPPSRDELTKNQVSLTCLVKGFYPSDIAVEWESNGQPENNYKTTPPVLDSDGSFFLYSKLTVDKSRWQQGNVFSCSVMHEGLHNHYTQKSLSLSPGK

SEQ ID NO: 4 - DNA, 549 bp, Artificial
  codon optimized sequence of (N-CCR4)3 protein DNA
atgaatccgaccgatattgcagataccacactggatgaaagcatctatagcaactattatctgtatgagagcattccgaaaccgtgtaccaaagaaggtattaaagcatttggcgaactgtttctgcctccgctgtatagcggtggtggtggtagtggtggcggtggttcaatgaacccgacagatatcgccgacacaaccctggatgaatcaatttattccaactactacctgtacgagtcaatcccgaaaccttgcacaaaagagggcatcaaagcctttggtgagctgtttttaccgcctctgtattcaggcggtggcggtagcggaggtggcggaagcatgaatcctacagacattgcggatacgaccctggacgagagcatttattcaaattactatttatacgaaagcatcccgaagccatgtacgaaagagggaattaaggcgttcggtgaattatttctgccaccgttatatagcttggatccgaattcgagctccgtcgacaagcttgcggccgcactcgagcaccaccaccaccaccac

SEQ ID NO: 5 - DNA, 1242 bp, Artificial
  (N-CCR4)3-Fc DNA
atggagacagacacactcctgctatgggtactgctgctctgggttccaggttccactggtgactcgatgaaccccaccgacatcgccgacaccaccctcgacgagagcatctacagcaactactacctgtacgaaagcatccccaaaccctgcaccaaagaaggcatcaaagccttcggcgagctgttcctcccccccctgtacagcggcggcggtggatctggcggcggaggatcaatgaaccccacagacatcgccgataccaccctggacgaaagcatttacagcaattactacctgtatgagtccatccccaaaccttgcaccaaagagggcatcaaggccttcggcgaactgttcctcccacccctgtacagtggcggcggcggaagcggaggcggaggaagcatgaaccccactgacatcgccgacacaaccctcgacgaaagcatatacagcaattattacctgtacgagtccatccctaaaccctgcacaaaggaaggcatcaaggcattcggagagctgttcctgccccccctgtatagcaagcttgacaaaactcacacatgcccaccgtgcccagcacctgaactcctggggggaccgtcagtcttcctcttccccccaaaacccaaggacaccctcatgatctcccggacccctgaggtcacatgcgtggtggtggacgtgagccacgaagaccctgaggtcaagttcaactggtacgtggacggcgtggaggtgcataatgccaagacaaagccgcgggaggagcagtacaacagcacgtaccgtgtggtcagcgtcctcaccgtcctgcaccaggactggctgaatggcaaggagtacaagtgcaaggtctccaacaaagccctcccagcccccatcgagaaaaccatctccaaagccaaagggcagccccgagaaccacaggtgtacaccctgcccccatcccgggatgagctgaccaagaaccaggtcagcctgacctgcctggtcaaaggcttctatcccagcgacatcgccgtggagtgggagagcaatgggcagccggagaacaactacaagaccacgcctcccgtgctggactccgacggctccttcttcctctacagcaagctcaccgtggacaagagcaggtggcagcaggggaacgtcttctcatgctccgtgatgcatgagggtctgcacaaccactacacgcagaagagcctctccctgtctccgggtaaataataa

SEQ ID NO: 6 - DNA, 885 bp, Artificial
  CCL22-GST DNA
atgggtccgtatggtgcaaatatggaagatagcgtttgttgccgtgattatgttcgttatcgtctgccgctgcgtgttgttaaacacttttattggaccagcgatagctgtccgcgtccgggtgttgttctgctgacctttcgtgataaagaaatttgtgcagatccgcgtgttccgtgggttaaaatgattctgaataaactgagccaggatccgggtggcccgggtatgtcccctatactaggttattggaaaattaagggccttgtgcaacccactcgacttcttttggaatatcttgaagaaaaatatgaagagcatttgtatgagcgcgatgaaggtgataaatggcgaaacaaaaagtttgaattgggtttggagtttcccaatcttccttattatattgatggtgatgttaaattaacacagtctatggccatcatacgttatatagctgacaagcacaacatgttgggtggttgtccaaaagagcgtgcagagatttcaatgcttgaaggagcggttttggatattagatacggtgtttcgagaattgcatatagtaaagactttgaaactctcaaagttgattttcttagcaagctacctgaaatgctgaaaatgttcgaagatcgtttatgtcataaaacatatttaaatggtgatcatgtaacccatcctgacttcatgttgtatgacgctcttgatgttgttttatacatggacccaatgtgcctggatgcgttcccaaaattagtttgttttaaaaaacgtattgaagctatcccacaaattgataagtacttgaaatccagcaagtatatagcatggcctttgcagggctggcaagccacgtttggtggtggcgaccatcctccaaaatga

SEQ ID NO: 7 - protein, 294 aa, Artificial
  CCL22-GST protein
MGPYGANMEDSVCCRDYVRYRLPLRVVKHFYWTSDSCPRPGVVLLTFRDKEICADPRVPWVKMILNKLSQDPGGPGMSPILGYWKIKGLVQPTRLLLEYLEEKYEEHLYERDEGDKWRNKKFELGLEFPNLPYYIDGDVKLTQSMAIIRYIADKHNMLGGCPKERAEISMLEGAVLDIRYGVSRIAYSKDFETLKVDFLSKLPEMLKMFEDRLCHKTYLNGDHVTHPDFMLYDALDVVLYMDPMCLDAFPKLVCFKKRIEAIPQIDKYLKSSKYIAWPLQGWQATFGGGDHPPK